European Patent Application EP 4 115 734 A1, published January 11, 2023. Title: Modified Plants Containing Combination of Apyrase Genes and Method for Making Modified Plants with Combination of Apyrase Genes. Applicant: Board of Regents, The University of Texas System. The sequence listing filed with the application follows.

SEQUENCE LISTING (4 sequences)

SEQ ID NO: 1 - protein, 455 aa, Pisum sativum
MELLIKLITFLLFSMPAITSSQYLGNNLLTSRKIFLKQEEISSYAVVFDAGSTGSRIHVYHFNQNLDLLHIGKGVEYYNKITPGLSSYANNPEQAAKSLIPLLEQAEDVVPDDLQPKTPVRLGATAGLRLLNGDASEKILQSVRDMLSNRSTFNVQPDAVSIIDGTQEGSYLWVTVNYALGNLGKKYTKTVGVIDLGGGSVQMAYAVSKKTAKNAPKVADGDDPYIKKVVLKGIPYDLYVHSYLHFGREASRAEILKLTPRSPNPCLLAGFNGIYTYSGEEFKATAYTSGANFNKCKNTIRKALKLNYPCPYQNCTFGGIWNGGGGNGQKNLFASSSFFYLPEDTGMVDASTPNFILRPVDIETKAKEACALNFEDAKSTYPFLDKKNVASYVCMDLIYQYVLLVDGFGLDPLQKITSGKEIEYQDAIVEAAWPLGNAVEAISALPKFERLMYFV

SEQ ID NO: 2 - protein, 455 aa, Artificial sequence
  Synthetic sequence
MELLIKLITFLLFSMPAITSSQYLGNNLLTSRKIFLKQEEISSYAVVFDAGSTGSRIHVYHFNQNLDLLHIGKGVEYYNKITPGLSSYANNPEQAAKSLIPLLEQAEDVVPDDLQPKTPVRLGATAGLRLLNGDASEKILQSVRDMLSNRSTFNVQPDAVSIIDGTQEGSYLWVTVNYALGNLGKKYTKTVGVIDLGGGSVQMAYAVLKKTAKNARKVADGDDPYIKKVVLKGIPYDLYVHSYLHFGREASRAEILKLTPRSPNPCLLAGFNGIYTYSGEEFKATAYTSGANFNKCKNTIRKALKLNYPCPYQNCTFGGIWNGGGGNGQKNLFASSSFFYLPEDTGMVDASTPNFILRPVDIETKAKEACALNFEDAKSTYPFLDKKNVASYVCMDLIYQYVLLVDGFGLDPLQKITSGKEIEYQDAIVEAAWPLGNAVEAISALPKFERLMYFV

SEQ ID NO: 3 - DNA, 1368 bp, Pisum sativum
atggagctccttattaaacttatcacttttctactattttctatgcctgcaatcacttcctcccaatacttaggaaacaacctactcaccagtagaaagattttcctaaaacaagaggaaatttcctcttacgctgtcgtattcgatgctggtagcactggtagtcgcattcatgtttaccattttaaccagaacttagatcttcttcatattggcaaaggtgtcgagtattataataagataacacctggtttgagttcatacgctaataatccagaacaggctgcaaaatctctcattccacttttagagcaagcagaagatgtcgtccccgacgatcttcaacccaagacacccgttagacttggggcaactgccggtttaaggcttttgaatggagatgcttctgaaaagatattgcaatcggtaagggatatgctgagcaacagaagtaccttcaacgttcaaccagacgcagtttctataattgatggaacccaagaaggttcttatctatgggtgacagttaactatgcattgggaaatttagggaaaaagtacacaaaaacagttggagtaatagatcttggaggtggatcagttcaaatggcgtatgcagtatcaaagaaaactgctaaaaatgctccaaaagttgcagatggagatgatccatacatcaagaaggttgtactcaagggaataccatatgatctctatgttcacagttacttacacttcggtagagaagcatctcgagcagagattttgaagctcactcctcgttctcctaacccttgccttttagctggatttaatggaatctatacatattcaggagaagagtttaaggcaactgcttacacttctggtgcaaactttaataaatgcaaaaacacaattcgtaaggctcttaagttgaactatccttgtccatatcagaattgcacttttggtggaatttggaatggtggaggaggaaatggacagaaaaacctttttgcttcttcatctttcttttacctacctgaagataccggtatggttgatgcaagcacacctaatttcatacttcggccggtcgatattgagactaaagctaaagaagcttgcgcgttaaacttcgaggatgcgaaatctacttatccatttcttgataagaaaaatgtagcttcatatgtatgcatggatcttatatatcagtatgtgttactcgttgatggatttggtcttgatccattgcaaaagattacatcagggaaggaaattgaataccaagatgctattgtggaagctgcatggcctctaggcaatgctgtagaagccatatcagctttacctaaatttgagcgattgatgtattttgtttaa

SEQ ID NO: 4 - DNA, 1368 bp, Artificial sequence
  Synthetic sequence
atggagctccttattaaacttatcacttttctactattttctatgcctgcaatcacttcctcccaatacttaggaaacaacctactcaccagtagaaagattttcctaaaacaagaggaaatttcctcttacgctgtcgtattcgatgctggtagcactggtagtcgcattcatgtttaccattttaaccagaacttagatcttcttcatattggcaaaggtgtcgagtattataataagataacacctggtttgagttcatacgctaataatccagaacaggctgcaaaatctctcattccacttttagagcaagcagaagatgtcgtccccgacgatcttcaacccaagacacccgttagacttggggcaactgccggtttaaggcttttgaatggagatgcttctgaaaagatattgcaatcggtaagggatatgctgagcaacagaagtaccttcaacgttcaaccagacgcagtttctataattgatggaacccaagaaggttcttatctatgggtgacagttaactatgcattgggaaatttagggaaaaagtacacaaaaacagttggagtaatagatcttggaggtggatcagttcaaatggcgtatgcagtattaaagaaaactgctaaaaatgctcgaaaagttgcagatggagatgatccatacatcaagaaggttgtactcaagggaataccatatgatctctatgttcacagttacttacacttcggtagagaagcatctcgagcagagattttgaagctcactcctcgttctcctaacccttgccttttagctggatttaatggaatctatacatattcaggagaagagtttaaggcaactgcttacacttctggtgcaaactttaataaatgcaaaaacacaattcgtaaggctcttaagttgaactatccttgtccatatcagaattgcacttttggtggaatttggaatggtggaggaggaaatggacagaaaaacctttttgcttcttcatctttcttttacctacctgaagataccggtatggttgatgcaagcacacctaatttcatacttcggccggtcgatattgagactaaagctaaagaagcttgcgcgttaaacttcgaggatgcgaaatctacttatccatttcttgataagaaaaatgtagcttcatatgtatgcatggatcttatatatcagtatgtgttactcgttgatggatttggtcttgatccattgcaaaagattacatcagggaaggaaattgaataccaagatgctattgtggaagctgcatggcctctaggcaatgctgtagaagccatatcagctttacctaaatttgagcgattgatgtattttgtttaa